European Patent Application EP 4 814 125 A2, published September 30, 2026. Title: ADENOVIRUSES AND METHODS FOR USING ADENOVIRUSES. Applicant: MAYO FOUNDATION FOR MEDICAL EDUCATION AND RESEARCH. Application US 62/770,631, filed November 21, 2018. The sequence listing filed with the application follows.

SEQUENCE LISTING (78 sequences)

SEQ ID NO: 1 - protein, 12 aa, synthetic construct
  REGION 1..12: note = targeting polypeptide
TARGEHKEEELI

SEQ ID NO: 2 - protein, 12 aa, synthetic construct
  REGION 1..12: note = targeting polypeptide
LRQTGAASAVWG

SEQ ID NO: 3 - protein, 12 aa, synthetic construct
  REGION 1..12: note = targeting polypeptide
ARRADTQWRGLE

SEQ ID NO: 4 - protein, 19 aa, synthetic construct
  REGION 1..19: note = targeting polypeptide
GTWLNPGFPPQSCGYATVT

SEQ ID NO: 5 - protein, 9 aa, synthetic construct
  REGION 1..9: note = targeting polypeptide
CDCRGDCFC

SEQ ID NO: 6 - protein, 10 aa, synthetic construct
  REGION 1..10: note = targeting polypeptide
NMSLDVNRKA

SEQ ID NO: 7 - protein, 12 aa, synthetic construct
  REGION 1..12: note = targeting polypeptide
ISLSSHRATWVV

SEQ ID NO: 8 - protein, 20 aa, synthetic construct
  REGION 1..20: note = targeting polypeptide
WTMGLDQLRDSSWAHGGFSA

SEQ ID NO: 9 - protein, 20 aa, synthetic construct
  REGION 1..20: note = targeting polypeptide
WTMGLDQLRGDSSWAHGGFS

SEQ ID NO: 10 - protein, 20 aa, synthetic construct
  REGION 1..20: note = targeting polypeptide
RSVSGTEWVPMNEQHRGAIW

SEQ ID NO: 11 - protein, 20 aa, synthetic construct
  REGION 1..20: note = targeting polypeptide
TELRTHTSKELTIRTAASSD

SEQ ID NO: 12 - protein, 20 aa, synthetic construct
  REGION 1..20: note = targeting polypeptide
DRAIGWQDKLYKLPLGSIHN

SEQ ID NO: 13 - protein, 20 aa, synthetic construct
  REGION 1..20: note = targeting polypeptide
MGSWEKAALWNRVSASSGGA

SEQ ID NO: 14 - protein, 20 aa, synthetic construct
  REGION 1..20: note = targeting polypeptide
MAMGGKPERPADSDNVQVRG

SEQ ID NO: 15 - protein, 20 aa, synthetic construct
  REGION 1..20: note = targeting polypeptide
MASRGDAGEGSTQSNTNVPS

SEQ ID NO: 16 - protein, 20 aa, synthetic construct
  REGION 1..20: note = targeting polypeptide
GPEDTSRAPENQQKTFHRRW

SEQ ID NO: 17 - protein, 20 aa, synthetic construct
  REGION 1..20: note = targeting polypeptide
MGREDVGEQKLISEEDLGGS

SEQ ID NO: 18 - protein, 11 aa, synthetic construct
  REGION 1..11: note = targeting polypeptide
ACDCRGDCFCG

SEQ ID NO: 19 - protein, 12 aa, synthetic construct
  REGION 1..12: note = targeting polypeptide
ACDCREDVCFCG

SEQ ID NO: 20 - protein, 20 aa, synthetic construct
  REGION 1..20: note = targeting polypeptide
GQIPITEPELCCVPWTEAFY

SEQ ID NO: 21 - protein, 20 aa, synthetic construct
  REGION 1..20: note = targeting polypeptide
PQPPNSTAHPNPHKAPPNTT

SEQ ID NO: 22 - protein, 20 aa, synthetic construct
  REGION 1..20: note = targeting polypeptide
VRWFPGGEWGVTHPESLPPP

SEQ ID NO: 23 - protein, 19 aa, synthetic construct
  REGION 1..19: note = targeting polypeptide
KKKKKKKKKKKKKKKKKKK

SEQ ID NO: 24 - protein, 14 aa, synthetic construct
  REGION 1..14: note = targeting polypeptide
GLNDIFEAQKIEWH

SEQ ID NO: 25 - protein, 23 aa, synthetic construct
  REGION 1..23: note = targeting polypeptide
CAAARWKKAFIAVSAANRFKKIS

SEQ ID NO: 26 - protein, 14 aa, synthetic construct
  REGION 1..14: note = targeting polypeptide
EDPGFFNVEIPEFP

SEQ ID NO: 27 - protein, 20 aa, synthetic construct
  REGION 1..20: note = targeting polypeptide
GGHGRVLWPDGWFSLVGISP

SEQ ID NO: 28 - protein, 21 aa, synthetic construct
  REGION 1..21: note = targeting polypeptide
MARTVTANVPGMGEGMVVVPC

SEQ ID NO: 29 - protein, 20 aa, synthetic construct
  REGION 1..20: note = targeting polypeptide
GVSKRGLQCHDFISCSGVPW

SEQ ID NO: 30 - protein, 20 aa, synthetic construct
  REGION 1..20: note = targeting polypeptide
NQSIPKVAGDSKVFCWWCAL

SEQ ID NO: 31 - protein, 20 aa, synthetic construct
  REGION 1..20: note = targeting polypeptide
QSTPPTKHLTIPRHLRNTLI

SEQ ID NO: 32 - protein, 20 aa, synthetic construct
  REGION 1..20: note = targeting polypeptide
DMSFQLVTPFLKALPTGWRG

SEQ ID NO: 33 - protein, 20 aa, synthetic construct
  REGION 1..20: note = targeting polypeptide
GGHGRVLWPDGWFSLVGISP

SEQ ID NO: 34 - protein, 8 aa, synthetic construct
  REGION 1..8: note = targeting polypeptide
FSLVGISP

SEQ ID NO: 35 - protein, 20 aa, synthetic construct
  REGION 1..20: note = targeting polypeptide
QIMMGPSLGYYMPSESIFAY

SEQ ID NO: 36 - protein, 20 aa, synthetic construct
  REGION 1..20: note = targeting polypeptide
ISWDIWRWWYTSEDRDAGSA

SEQ ID NO: 37 - protein, 20 aa, synthetic construct
  REGION 1..20: note = targeting polypeptide
VWGMTTSDHQRKTERLDSPE

SEQ ID NO: 38 - protein, 20 aa, synthetic construct
  REGION 1..20: note = targeting polypeptide
MTSAQTSEKLKAETDRHTAE

SEQ ID NO: 39 - protein, 19 aa, synthetic construct
  REGION 1..19: note = targeting polypeptide
MGSRSAVGDFESAEGSRRP

SEQ ID NO: 40 - protein, 20 aa, synthetic construct
  REGION 1..20: note = targeting polypeptide
MGRTVQSGDGTPAQTQPSVN

SEQ ID NO: 41 - protein, 20 aa, synthetic construct
  REGION 1..20: note = targeting polypeptide
MARTVTANVPGMGEGMVVVP

SEQ ID NO: 42 - protein, 132 aa, synthetic construct
  REGION 1..132: note = Adenovirus E1A N-terminus polypeptide
MRHIICHGGVITEEMAASLLDQLIEEVLADNLPPPSHFEPPTLHELYDLDVTAPEDPNEEAVSQIFPESVMLAVQEGIDLFTFPPAPGSPEPPHLSRQPEQPEQRALGPVSMPNLVPEVIDLTCHEAGFPPS

SEQ ID NO: 43 - protein, 112 aa, synthetic construct
  REGION 1..112: note = E1A N-terminus polypeptide
MRHIEEVLADNLPPPSHFEPPTLHELYDLDVTAPEDPNEEAVSQIFPESVMLAVQEGIDLFTFPPAPGSPEPPHLSRQPEQPEQRALGPVSMPNLVPEVIDLTCHEAGFPPS

SEQ ID NO: 44 - protein, 119 aa, synthetic construct
  REGION 1..119: note = E1A N-terminus polypeptide
MRHIICHGGVITEEMAASLLDQLIEEVLADNLPPPSHFEPPTLHELYDLDVTAPEDPNEEAVSQIFPESVMLAVQEGIDLFTFPPAPGSPEPPHLSRQPEQPEQRALGPVCHEAGFPPS

SEQ ID NO: 45 - protein, 99 aa, synthetic construct
  REGION 1..99: note = E1A N-terminus polypeptide
MRHIEEVLADNLPPPSHFEPPTLHELYDLDVTAPEDPNEEAVSQIFPESVMLAVQEGIDLFTFPPAPGSPEPPHLSRQPEQPEQRALGPVCHEAGFPPS

SEQ ID NO: 46 - protein, 5 aa, synthetic construct
  REGION 1..5: note = Cell Binding Peptide
REDVY

SEQ ID NO: 47 - protein, 12 aa, synthetic construct
  REGION 1..12: note = Breast Cancer Binding Peptide
ISLSSHRATWVV

SEQ ID NO: 48 - protein, 1608 aa, synthetic construct
  REGION 1..1608: note = Probasin-E1 nucleic acid
TCGAGCGACGGTATCGATAAGCTTGGAGCTTATGATAGCATCTTGTTCTTAGTCTTTTTCTTAATAGGGACATAAAGCCCACAAATAAAAATATGCCTGAAGAATGGGACAGGCATTGGGCATTGTCCATGCCTAGTAAAGTACTCCAAGAACCTATTTGTATACTAGATGACACAATGTTCTAGCCAAGCTTGGTAGTCATCATGTTTAAACATCTACCATTCCAGTTAAGAAAATATGATAGCATCTTGTTCTTAGTCTTTTTCTTAATAGGGACATAAAGCCCACAAATAAAAATATGCCTGAAGAATGGGACAGGCATTGGGCATTGTCCATGCCTAGTAAAGTACTCCAAGAACCTATTTGTATACTAGATGACACAATGTCAATGTCTGTGTACAACTGCCAACTGGGATGCAAGACACTGCCCATGCCAATCATCCTGAAAAGCAGCTATAAAAAGCAGGAAGCTACTCTGCACCTTGTCAGTGAGGTCCAGATACCTCCCTCGAGCGGCCGCGACGCGCAGTGTATTTATACCCGGTGAGTTCCTCAAGAGGCCACTCTTGAGTGCCAGCGAGTAGAGTTTTCTCCTCCGAGCCGCTCCGACACCGGGACTGAAAATGAGACATATTATCTGCCACGGAGGTGTTATTACCGAAGAAATGGCCGCCAGTCTTTTGGACCAGCTGATCGAAGAGGTACTGGCTGATAATCTTCCACCTCCTAGCCATTTTGAACCACCTACCCTTCACGAACTGTATGATTTAGACGTGACGGCCCCCGAAGATCCCAACGAGGAGGCGGTTTCGCAGATTTTTCCCGAGTCTGTAATGTTGGCGGTGCAGGAAGGGATTGACTTATTCACTTTTCCGCCGGCGCCCGGTTCTCCGGAGCCGCCTCACCTTTCCCGGCAGCCCGAGCAGCCGGAGCAGAGAGCCTTGGGTCCGGTTTCTATGCCAAACCTTGTGCCGGAGGTGATCGATCTTACCTGCCACGAGGCTGGCTTTCCACCCAGTGACGACGAGGATGAAGAGGGTGAGGAGTTTGTGTTAGATTATGTGGAGCACCCCGGGCACGGTTGCAGGTCTTGTCATTATCACCGGAGGAATACGGGGGACCCAGATATTATGTGTTCGCTTTGCTATATGAGGACCTGTGGCATGTTTGTCTACAGTAAGTGAAAATTATGGGCAGTCGGTGATAGAGTGGTGGGTTTGGTGTGGTAATTTTTTTTTAATTTTTACAGTTTTGTGGTTTAAAGAATTTTGTATTGTGATTTTTTAAAAGGTCCTGTGTCTGAACCTGAGCCTGAGCCCGAGCCAGAACCGGAGCCTGCAAGACCTACCCGGCGTCCTAAATTGGTGCCTGCTATCCTGAGACGCCCGACATCACCTGTGTCTAGAGAATGCAATAGTAGTACGGATAGCTGTGACTCCGGTCCTTCTAACACACCTCCTGAGATACACCCGGTGGTCCCGCTGTGCCCCATTAAACCAGTTGCCGTGAGAGTTGGTGGGCGTCGCCAGGCTGTGGAATGTATCGAGGACTTGCTTAACGAGTCTGGGCAACCTTTGGACTTGAGCTGTAAACGCCCCAGGCCATAAG

SEQ ID NO: 49 - protein, 959 aa, synthetic construct
  REGION 1..959: note = Hexon Polypeptide
MATPSMMPQWSYMHISGQDASEYLSPGLVQFARATETYFSLNNKFRNPTVAPTHDVTTDRSQRLTLRFIPVDREDTAYSYKARFTLAVGDNRVLDMASTYFDIRGVLDRGPTFKPYSGTAYNALAPKGAPNSCEWDEDDTQVQVAAEDDQDDDEEEEQLPQQRNGKKTHVYAQAPFAGEAINKNGLQIGTNGAATEGNKEIYADKTYQPEPQIGESQWNEAESSVAGGRVLKKTTPMKPCYGSYARPTNSNGGQGVMVEQNGKLESQVEMQFFSTSVNAMNEANAIQPKLVLYSEDVNMETPDTHLSYKPGKSDDNSKAMLGQQSMPNRPNYIAFRDNFIGLMYYNSTGNMGVLAGQASQLNAVVDLQDRNTELSYQLLLDSIGDRTRYFSMWNQAVDSYDPDVRIIENHGTEDELPNYCFPLGGIGVTDTYQAIKATNGNGGATTWAQDNTFAERNEIGVGNNFAMEINLNANLWRNFLYSNIALYLPDKLKYNPTNVEISDNPNTYDYMNKRVVAPGLVDCYINLGARWSLDYMDNVNPFNHHRNAGLRYRSMLLGNGRYVPFHIQVPQKFFAIKNLLLLPGSYTYEWNFRKDVNMVLQSSLGNDLRVDGASIKFDSICLYATFFPMAHNTASTLEAMLRNDTNDQSFNDYLSAANMLYPIPANATNVPISIPSRNWAAFRGWAFTRLKTKETPSLGSGYDPYYTYSGSIPYLDGTFYLNHTFKKVAITFDSSVSWPGNDRLLTPNEFEIKRSVDGEGYNVAQCNMTKDWFLVQMLANYNIGYQGFYIPESYKDRMYSFFRNFQPMSRQVVDDTKYKDYQQVGIIHQHNNSGFVGYLAPTMREGQAYPANVPYPLIGKTAVDSITQKKFLCDRTLWRIPFSSNFMSMGALTDLGQNLLYANSAHALDMTFEVDPMDEPTLLYVLFEVFDVVRVHQPHRGVIETVYLRTPFSAGNATT

SEQ ID NO: 50 - protein, 967 aa, synthetic construct
  REGION 1..967: note = Hexon Polypeptide
MATPSMMPQWSYMHISGQDASEYLSPGLVQFARATETYFSLNNKFRNPTVAPTHDVTTDRSQRLTLRFIPVDREDTAYSYKARFTLAVGDNRVLDMASTYFDIRGVLDRGPTFKPYSGTAYNALAPKGAPNSCEWDEDDTQVQVAAEDDQDDDSSCSSGGTEEEEQLPQQRNGKKTHVYAQAPFAGEAINKNGLQIGTNGAATEGNKEIYADKTYQPEPQIGESQWNEAESSVAGGRVLKKTTPMKPCYGSYARPTNSNGGQGVMVEQNGKLESQVEMQFFSTSVNAMNEANAIQPKLVLYSEDVNMETPDTHLSYKPGKSDDNSKAMLGQQSMPNRPNYIAFRDNFIGLMYYNSTGNMGVLAGQASQLNAVVDLQDRNTELSYQLLLDSIGDRTRYFSMWNQAVDSYDPDVRIIENHGTEDELPNYCFPLGGIGVTDTYQAIKATNGNGGATTWAQDNTFAERNEIGVGNNFAMEINLNANLWRNFLYSNIALYLPDKLKYNPTNVEISDNPNTYDYMNKRVVAPGLVDCYINLGARWSLDYMDNVNPFNHHRNAGLRYRSMLLGNGRYVPFHIQVPQKFFAIKNLLLLPGSYTYEWNFRKDVNMVLQSSLGNDLRVDGASIKFDSICLYATFFPMAHNTASTLEAMLRNDTNDQSFNDYLSAANMLYPIPANATNVPISIPSRNWAAFRGWAFTRLKTKETPSLGSGYDPYYTYSGSIPYLDGTFYLNHTFKKVAITFDSSVSWPGNDRLLTPNEFEIKRSVDGEGYNVAQCNMTKDWFLVQMLANYNIGYQGFYIPESYKDRMYSFFRNFQPMSRQVVDDTKYKDYQQVGIIHQHNNSGFVGYLAPTMREGQAYPANVPYPLIGKTAVDSITQKKFLCDRTLWRIPFSSNFMSMGALTDLGQNLLYANSAHALDMTFEVDPMDEPTLLYVLFEVFDVVRVHQPHRGVIETVYLRTPFSAGNATT

SEQ ID NO: 51 - protein, 955 aa, synthetic construct
  REGION 1..955: note = Hexon Polypeptide
MATPSMMPQWSYMHISGQDASEYLSPGLVQFARATETYFSLNNKFRNPTVAPTHDVTTDRSQRLTLRFIPVDREDTAYSYKARFTLAVGDNRVLDMASTYFDIRGVLDRGPTFKPYSGTAYNALAPKGAPNSCEWDEDDTQVQVAAEDDQDDDEEEEQLPQQRNGKKTHVYAQAPFAGEAINKNGLQIGTNGAATEGNKEIYADKTYQPEPQIGESQWNEAESSVAGGRVLKKTTPMKPCYGSYARPTNSNGGQGVMVEQNGKLESQVEMQFFSTSSCSSGGTPKLVLYSEDVNMETPDTHLSYKPGKSDDNSKAMLGQQSMPNRPNYIAFRDNFIGLMYYNSTGNMGVLAGQASQLNAVVDLQDRNTELSYQLLLDSIGDRTRYFSMWNQAVDSYDPDVRIIENHGTEDELPNYCFPLGGIGVTDTYQAIKATNGNGGATTWAQDNTFAERNEIGVGNNFAMEINLNANLWRNFLYSNIALYLPDKLKYNPTNVEISDNPNTYDYMNKRVVAPGLVDCYINLGARWSLDYMDNVNPFNHHRNAGLRYRSMLLGNGRYVPFHIQVPQKFFAIKNLLLLPGSYTYEWNFRKDVNMVLQSSLGNDLRVDGASIKFDSICLYATFFPMAHNTASTLEAMLRNDTNDQSFNDYLSAANMLYPIPANATNVPISIPSRNWAAFRGWAFTRLKTKETPSLGSGYDPYYTYSGSIPYLDGTFYLNHTFKKVAITFDSSVSWPGNDRLLTPNEFEIKRSVDGEGYNVAQCNMTKDWFLVQMLANYNIGYQGFYIPESYKDRMYSFFRNFQPMSRQVVDDTKYKDYQQVGIIHQHNNSGFVGYLAPTMREGQAYPANVPYPLIGKTAVDSITQKKFLCDRTLWRIPFSSNFMSMGALTDLGQNLLYANSAHALDMTFEVDPMDEPTLLYVLFEVFDVVRVHQPHRGVIETVYLRTPFSAGNATT

SEQ ID NO: 52 - protein, 964 aa, synthetic construct
  REGION 1..964: note = Hexon Polypeptide
MATPSMMPQWSYMHISGQDASEYLSPGLVQFARATETYFSLNNKFRNPTVAPTHDVTTDRSQRLTLRFIPVDREDTAYSYKARFTLAVGDNRVLDMASTYFDIRGVLDRGPTFKPYSGTAYNALAPKGAPNSCEWDEDDTQVQVAAEDDQDDDSSGGTEEEEQLPQQRNGKKTHVYAQAPFAGEAINKNGLQIGTNGAATEGNKEIYADKTYQPEPQIGESQWNEAESSVAGGRVLKKTTPMKPCYGSYARPTNSNGGQGVMVEQNGKLESQVEMQFFSTSVNAMNEANAIQPKLVLYSEDVNMETPDTHLSYKPGKSDDNSKAMLGQQSMPNRPNYIAFRDNFIGLMYYNSTGNMGVLAGQASQLNAVVDLQDRNTELSYQLLLDSIGDRTRYFSMWNQAVDSYDPDVRIIENHGTEDELPNYCFPLGGIGVTDTYQAIKATNGNGGATTWAQDNTFAERNEIGVGNNFAMEINLNANLWRNFLYSNIALYLPDKLKYNPTNVEISDNPNTYDYMNKRVVAPGLVDCYINLGARWSLDYMDNVNPFNHHRNAGLRYRSMLLGNGRYVPFHIQVPQKFFAIKNLLLLPGSYTYEWNFRKDVNMVLQSSLGNDLRVDGASIKFDSICLYATFFPMAHNTASTLEAMLRNDTNDQSFNDYLSAANMLYPIPANATNVPISIPSRNWAAFRGWAFTRLKTKETPSLGSGYDPYYTYSGSIPYLDGTFYLNHTFKKVAITFDSSVSWPGNDRLLTPNEFEIKRSVDGEGYNVAQCNMTKDWFLVQMLANYNIGYQGFYIPESYKDRMYSFFRNFQPMSRQVVDDTKYKDYQQVGIIHQHNNSGFVGYLAPTMREGQAYPANVPYPLIGKTAVDSITQKKFLCDRTLWRIPFSSNFMSMGALTDLGQNLLYANSAHALDMTFEVDPMDEPTLLYVLFEVFDVVRVHQPHRGVIETVYLRTPFSAGNATT

SEQ ID NO: 53 - protein, 952 aa, synthetic construct
  REGION 1..952: note = Hexon Polypeptide
MATPSMMPQWSYMHISGQDASEYLSPGLVQFARATETYFSLNNKFRNPTVAPTHDVTTDRSQRLTLRFIPVDREDTAYSYKARFTLAVGDNRVLDMASTYFDIRGVLDRGPTFKPYSGTAYNALAPKGAPNSCEWDEDDTQVQVAAEDDQDDDEEEEQLPQQRNGKKTHVYAQAPFAGEAINKNGLQIGTNGAATEGNKEIYADKTYQPEPQIGESQWNEAESSVAGGRVLKKTTPMKPCYGSYARPTNSNGGQGVMVEQNGKLESQVEMQFFSTSSGGTPKLVLYSEDVNMETPDTHLSYKPGKSDDNSKAMLGQQSMPNRPNYIAFRDNFIGLMYYNSTGNMGVLAGQASQLNAVVDLQDRNTELSYQLLLDSIGDRTRYFSMWNQAVDSYDPDVRIIENHGTEDELPNYCFPLGGIGVTDTYQAIKATNGNGGATTWAQDNTFAERNEIGVGNNFAMEINLNANLWRNFLYSNIALYLPDKLKYNPTNVEISDNPNTYDYMNKRVVAPGLVDCYINLGARWSLDYMDNVNPFNHHRNAGLRYRSMLLGNGRYVPFHIQVPQKFFAIKNLLLLPGSYTYEWNFRKDVNMVLQSSLGNDLRVDGASIKFDSICLYATFFPMAHNTASTLEAMLRNDTNDQSFNDYLSAANMLYPIPANATNVPISIPSRNWAAFRGWAFTRLKTKETPSLGSGYDPYYTYSGSIPYLDGTFYLNHTFKKVAITFDSSVSWPGNDRLLTPNEFEIKRSVDGEGYNVAQCNMTKDWFLVQMLANYNIGYQGFYIPESYKDRMYSFFRNFQPMSRQVVDDTKYKDYQQVGIIHQHNNSGFVGYLAPTMREGQAYPANVPYPLIGKTAVDSITQKKFLCDRTLWRIPFSSNFMSMGALTDLGQNLLYANSAHALDMTFEVDPMDEPTLLYVLFEVFDVVRVHQPHRGVIETVYLRTPFSAGNATT

SEQ ID NO: 54 - protein, 1033 aa, synthetic construct
  REGION 1..1033: note = Hexon Polypeptide
MATPSMMPQWSYMHISGQDASEYLSPGLVQFARATETYFSLNNKFRNPTVAPTHDVTTDRSQRLTLRFIPVDREDTAYSYKARFTLAVGDNRVLDMASTYFDIRGVLDRGPTFKPYSGTAYNALAPKGAPNSCEWDEDDTQVQVAAEDDQDDDSTGEIPAPLAGTVSKILVKEGDTVKAGQTVLVLEAMKMETEINAPTDGKVEKVLVKERDAVQGGQGLIKIGGGTEEEEQLPQQRNGKKTHVYAQAPFAGEAINKNGLQIGTNGAATEGNKEIYADKTYQPEPQIGESQWNEAESSVAGGRVLKKTTPMKPCYGSYARPTNSNGGQGVMVEQNGKLESQVEMQFFSTSVNAMNEANAIQPKLVLYSEDVNMETPDTHLSYKPGKSDDNSKAMLGQQSMPNRPNYIAFRDNFIGLMYYNSTGNMGVLAGQASQLNAVVDLQDRNTELSYQLLLDSIGDRTRYFSMWNQAVDSYDPDVRIIENHGTEDELPNYCFPLGGIGVTDTYQAIKATNGNGGATTWAQDNTFAERNEIGVGNNFAMEINLNANLWRNFLYSNIALYLPDKLKYNPTNVEISDNPNTYDYMNKRVVAPGLVDCYINLGARWSLDYMDNVNPFNHHRNAGLRYRSMLLGNGRYVPFHIQVPQKFFAIKNLLLLPGSYTYEWNFRKDVNMVLQSSLGNDLRVDGASIKFDSICLYATFFPMAHNTASTLEAMLRNDTNDQSFNDYLSAANMLYPIPANATNVPISIPSRNWAAFRGWAFTRLKTKETPSLGSGYDPYYTYSGSIPYLDGTFYLNHTFKKVAITFDSSVSWPGNDRLLTPNEFEIKRSVDGEGYNVAQCNMTKDWFLVQMLANYNIGYQGFYIPESYKDRMYSFFRNFQPMSRQVVDDTKYKDYQQVGIIHQHNNSGFVGYLAPTMREGQAYPANVPYPLIGKTAVDSITQKKFLCDRTLWRIPFSSNFMSMGALTDLGQNLLYANSAHALDMTFEVDPMDEPTLLYVLFEVFDVVRVHQPHRGVIETVYLRTPFSAGNATT

SEQ ID NO: 55 - protein, 1021 aa, synthetic construct
  REGION 1..1021: note = Hexon Polypeptide
MATPSMMPQWSYMHISGQDASEYLSPGLVQFARATETYFSLNNKFRNPTVAPTHDVTTDRSQRLTLRFIPVDREDTAYSYKARFTLAVGDNRVLDMASTYFDIRGVLDRGPTFKPYSGTAYNALAPKGAPNSCEWDEDDTQVQVAAEDDQDDDEEEEQLPQQRNGKKTHVYAQAPFAGEAINKNGLQIGTNGAATEGNKEIYADKTYQPEPQIGESQWNEAESSVAGGRVLKKTTPMKPCYGSYARPTNSNGGQGVMVEQNGKLESQVEMQFFSTSTGEIPAPLAGTVSKILVKEGDTVKAGQTVLVLEAMKMETEINAPTDGKVEKVLVKERDAVQGGQGLIKIGGGTPKLVLYSEDVNMETPDTHLSYKPGKSDDNSKAMLGQQSMPNRPNYIAFRDNFIGLMYYNSTGNMGVLAGQASQLNAVVDLQDRNTELSYQLLLDSIGDRTRYFSMWNQAVDSYDPDVRIIENHGTEDELPNYCFPLGGIGVTDTYQAIKATNGNGGATTWAQDNTFAERNEIGVGNNFAMEINLNANLWRNFLYSNIALYLPDKLKYNPTNVEISDNPNTYDYMNKRVVAPGLVDCYINLGARWSLDYMDNVNPFNHHRNAGLRYRSMLLGNGRYVPFHIQVPQKFFAIKNLLLLPGSYTYEWNFRKDVNMVLQSSLGNDLRVDGASIKFDSICLYATFFPMAHNTASTLEAMLRNDTNDQSFNDYLSAANMLYPIPANATNVPISIPSRNWAAFRGWAFTRLKTKETPSLGSGYDPYYTYSGSIPYLDGTFYLNHTFKKVAITFDSSVSWPGNDRLLTPNEFEIKRSVDGEGYNVAQCNMTKDWFLVQMLANYNIGYQGFYIPESYKDRMYSFFRNFQPMSRQVVDDTKYKDYQQVGIIHQHNNSGFVGYLAPTMREGQAYPANVPYPLIGKTAVDSITQKKFLCDRTLWRIPFSSNFMSMGALTDLGQNLLYANSAHALDMTFEVDPMDEPTLLYVLFEVFDVVRVHQPHRGVIETVYLRTPFSAGNATT

SEQ ID NO: 56 - protein, 1015 aa, synthetic construct
  REGION 1..1015: note = Hexon Polypeptide
MATPSMMPQWSYMHISGQDASEYLSPGLVQFARATETYFSLNNKFRNPTVAPTHDVTTDRSQRLTLRFIPVDREDTAYSYKARFTLAVGDNRVLDMASTYFDIRGVLDRGPTFKPYSGTAYNALAPKGAPNSCEWDEDDTQVQVAAEDDQDDDEEEEQLPQQRNGKKTHVYAQAPFAGEAINKNGLQIGTNGAATEGNKEIYADKTYQPEPQIGESQWNEAESSVAGGRVLKKTTPMKPCYGSYARPTNSNGGQGVMVEQNGKLESQVEMQFFSTSSSNFTREGNVTYKEEMDKVKNCSFNVTTGIRDKKQKVNALFYRLDITPLDENNNNSSEYRLINSGGTPKLVLYSEDVNMETPDTHLSYKPGKSDDNSKAMLGQQSMPNRPNYIAFRDNFIGLMYYNSTGNMGVLAGQASQLNAVVDLQDRNTELSYQLLLDSIGDRTRYFSMWNQAVDSYDPDVRIIENHGTEDELPNYCFPLGGIGVTDTYQAIKATNGNGGATTWAQDNTFAERNEIGVGNNFAMEINLNANLWRNFLYSNIALYLPDKLKYNPTNVEISDNPNTYDYMNKRVVAPGLVDCYINLGARWSLDYMDNVNPFNHHRNAGLRYRSMLLGNGRYVPFHIQVPQKFFAIKNLLLLPGSYTYEWNFRKDVNMVLQSSLGNDLRVDGASIKFDSICLYATFFPMAHNTASTLEAMLRNDTNDQSFNDYLSAANMLYPIPANATNVPISIPSRNWAAFRGWAFTRLKTKETPSLGSGYDPYYTYSGSIPYLDGTFYLNHTFKKVAITFDSSVSWPGNDRLLTPNEFEIKRSVDGEGYNVAQCNMTKDWFLVQMLANYNIGYQGFYIPESYKDRMYSFFRNFQPMSRQVVDDTKYKDYQQVGIIHQHNNSGFVGYLAPTMREGQAYPANVPYPLIGKTAVDSITQKKFLCDRTLWRIPFSSNFMSMGALTDLGQNLLYANSAHALDMTFEVDPMDEPTLLYVLFEVFDVVRVHQPHRGVIETVYLRTPFSAGNATT

SEQ ID NO: 57 - protein, 987 aa, synthetic construct
  REGION 1..987: note = Hexon Polypeptide
MATPSMMPQWSYMHISGQDASEYLSPGLVQFARATETYFSLNNKFRNPTVAPTHDVTTDRSQRLTLRFIPVDREDTAYSYKARFTLAVGDNRVLDMASTYFDIRGVLDRGPTFKPYSGTAYNALAPKGAPNSCEWDEDDTQVQVAAEDDQDDDEEEEQLPQQRNGKKTHVYAQAPFAGEAINKNGLQIGTNGAATEGNKEIYADKTYQPEPQIGESQWNEAESSVAGGRVLKKTTPMKPCYGSYARPTNSNGGQGVMVEQNGKLESQVEMQFFSTSSQAEPDRAHYNIVTFCCKCDQLLRREVYDFAFRDLSGGTPKLVLYSEDVNMETPDTHLSYKPGKSDDNSKAMLGQQSMPNRPNYIAFRDNFIGLMYYNSTGNMGVLAGQASQLNAVVDLQDRNTELSYQLLLDSIGDRTRYFSMWNQAVDSYDPDVRIIENHGTEDELPNYCFPLGGIGVTDTYQAIKATNGNGGATTWAQDNTFAERNEIGVGNNFAMEINLNANLWRNFLYSNIALYLPDKLKYNPTNVEISDNPNTYDYMNKRVVAPGLVDCYINLGARWSLDYMDNVNPFNHHRNAGLRYRSMLLGNGRYVPFHIQVPQKFFAIKNLLLLPGSYTYEWNFRKDVNMVLQSSLGNDLRVDGASIKFDSICLYATFFPMAHNTASTLEAMLRNDTNDQSFNDYLSAANMLYPIPANATNVPISIPSRNWAAFRGWAFTRLKTKETPSLGSGYDPYYTYSGSIPYLDGTFYLNHTFKKVAITFDSSVSWPGNDRLLTPNEFEIKRSVDGEGYNVAQCNMTKDWFLVQMLANYNIGYQGFYIPESYKDRMYSFFRNFQPMSRQVVDDTKYKDYQQVGIIHQHNNSGFVGYLAPTMREGQAYPANVPYPLIGKTAVDSITQKKFLCDRTLWRIPFSSNFMSMGALTDLGQNLLYANSAHALDMTFEVDPMDEPTLLYVLFEVFDVVRVHQPHRGVIETVYLRTPFSAGNATT

SEQ ID NO: 58 - protein, 959 aa, synthetic construct; identical to SEQ ID NO: 49
  REGION 1..959: note = Hexon Polypeptide

SEQ ID NO: 59 - protein, 962 aa, synthetic construct
  REGION 1..962: note = Hexon Polypeptide
MATPSMMPQWSYMHISGQDASEYLSPGLVQFARATETYFSLNNKFRNPTVAPTHDVTTDRSQRLTLRFIPVDREDTAYSYKARFTLAVGDNRVLDMASTYFDIRGVLDRGPTFKPYSGTAYNALAPKGAPNSCEWEQNETAQVDAQELDEEENEANEAQAREQEQAKKTHVYAQAPLSGEAINKNGLQIGTNGAATEGNKEIYADKTYQPEPQIGESQWNEAESSVAGGRVLKKTTPMKPCYGSYARPTNSNGGQGVMVEQNGKLESQVEMQFFSTSVNAMNEANAIQPKLVLYSEDVNMETPDTHLSYKPGKSDDNSKAMLGQQSMPNRPNYIAFRDNFIGLMYYNSTGNMGVLAGQASQLNAVVDLQDRNTELSYQLLLDSIGDRTRYFSMWNQAVDSYDPDVRIIENHGTEDELPNYCFPLGGIGITDTFQAVKTTAANGDQGNTTWQKDSTFAERNEIGVGNNFAMEINLNANLWRNFLYSNIALYLPDKLKYNPTNVEISDNPNTYDYMNKRVVAPGLVDCYINLGARWSLDYMDNVNPFNHPRHAGLRYRSMLLGNGRYVPFHIQVPQKFFAIKNLLLLPGSYTYEWNFRKDVNMVLQSSLGNDLRVDGASIKFDSICLYATFFPMAHNTASTLEAMLRNDTNDQSFNDYLSAANMLYPIPANATNVPISIPSRNWAAFRGWAFTRLKTKETPSLGSGYDPYYTYSGSIPYLDGTFYLNHTFKKVAITFDSSVSWPGNDRLLTPNEFEIKRSVDGEGYNVAQCNMTKDWFLVQMLANYNIGYQGFYIPESYKDRMYSFFRNFQPMSRQVVDDTKYKDYQQVGIIHQHNNSGFVGYLAPTMREGQAYPANVPYPLIGKTAVDSITQKKFLCDRTLWRIPFSSNFMSMGALTDLGQNLLYANSAHALDMTFEVDPMDEPTLLYVLFEVFDVVRVHQPHRGVIETVYLRTPFSAGNATT

SEQ ID NO: 60 - protein, 528 aa, synthetic construct
  REGION 1..528: note = Fiber Polypeptide
MKRARPSEDTFNPVYPYDTETGPPTVPFLTPPFVSPNGFQESPPGVLSLRLSEPLVTSHGMLALKMGSGLSLDQAGNLTSNTITVSQPLKKTKSNITLETSAPLTVSSGALTMATTSPLVVSDNTLTMQSQAPLTVQDSKLSIATKEPLTVLDGKLALQTSAPLSATDNNALTITASPPLTTANGSLAVTMENPLYNNNGKLGLKIGGPLQVATDSHALTLGTGQGVAVHNNLLHTKVTGAIGFDTSGNMELKTGDGLYVDSAGPNQKLHINLNTTKGLAFDNTAITINAGKGLEFETDSSNGNPIKTKIGSGIQYNTNGAMVAKLGTGLSFDSSGAITMGSINNDRLTLWTTPDPSPNCRIASDKDCKLTLALTKCGSQILGTVSALAVSGNMASINGTLSSVNLVLRFDDNGVLMSNSSLDKQYWNFRNGDSTNGQPYTYAVGFMPNLKAYPKTQSKTAKSNIVSQVYLNGDKSKPLHFTITLNGTDETNQVSKYSISFSWSWNSGQYTNDKFATNSYTFSYIAQE

SEQ ID NO: 61 - protein, 324 aa, synthetic construct
  REGION 1..324: note = Fiber Polypeptide
MKRARPSEDTFNPVYPYDTETGPPTVPFLTPPFVSPNGFQESPPGVLTLKCLTPLTTTGGSLQLKVGGGLTVDDTDGTLQENIRATAPITKNNHSVELSIGNGLETQNNKLCAKLGNGLKFNNGDICIKDSINTLWTGINPPPNCQIVENTNTNDGKLTLVLVKNGGLVNGYVSLVGVSDTVNQMFTQKTANIQLRLYFDSSGNLLTDESDLKIPLKNKSSTATSETVASSKAFMPSTTAYPFNTTTRDSENYIHGICYYMTSYDRSLFPLNISIMLNSRMISSNVAYAIQFEWNLNASESPESNIATLTTSPFFFSYITEDDN

SEQ ID NO: 62 - protein, 534 aa, synthetic construct
  REGION 1..534: note = Fiber Polypeptide
MKRARPSEDTFNPVYPYDTETGPPTVPFLTPPFVSPNGFQESPPGVLSLRLSEPLVTSHGMLALKMGSGLSLDQAGNLTSNTITVSQPLKKTKSNITLETSAPLTVSSGALTMATTSPLVVSDNTLTMQSQAPLTVQDSKLSIATKEPLTVLDGKLALQTSAPLSATDNNALTITASPPLTTANGSLAVTMENPLYNNNGKLGLKIGGPLQVATDSHALTLGTGQGVAVHNNLLHTKVTGAIGFDTSGNMELKTGDGLYVDSAGPNQKLHINLNTTKGLAFDNTAITINAGKGLEFETDSSNGNPIKTKIGSGIQYNTNGAMVAKLGTGLSFDSSGAITMGSINNDRLTLWTTPDPSPNCRIASDKDCKLTLALTKCGSQILGTVSALAVSGNMASINGTLSSVNLVLRFDDNGVLMSNSSLDKQYWNFRNGDSTNGQPYTYAVGFMPNLKAYPKTQSKTAKSNIVSQVYLNGDKSKPLHFTITLNGTDETNQVSKYSISFSWSWNSGQYTNDKFATNSYTFSYIAQEKKKKKK

SEQ ID NO: 63 - protein, 425 aa, synthetic construct
  REGION 1..425: note = Fiber Polypeptide
MKRARPSEDTFNPVYPYDTETGPPTVPFLTPPFVSPNGFQESPPGVLSLRLSEPLVTKNGEITLKLGEGVDLDSSGKLISNTATKAAAPLSFSNNTISLNMDHPFYTKDGKLSLQVSPPLNILRTSILNTLALGFGSGLGLRGSALAVQLVSPLTFDTDGNIKLTLDRGLHVTTGDAIESNISWAKGLKFEDGAIATNIGNGLEFGSSSTETGVDDAYPIQVKLGSGLSFDSTGAIMAGNKEDDKLTLWTTPDPSPNCQILAENDAKLTLCLTKCGSQILATVSVLVVGSGNLNPITGTVSSAQVFLRFDANGVLLTEHSTLKKYWGYRQGDSIDGTPYTNAVGFMPNLKAYPKSQSSTTKNNIVGQVYMNGDVSKPMLLTITLNGTDDSNSTYSMSFSYTWTNGSYVGATFGANSYTFSYIAQE

SEQ ID NO: 64 - protein, 432 aa, synthetic construct
  REGION 1..432: note = Fiber Polypeptide
MKRARPSEDTFNPVYPYDTETGPPTVPFLTPPFVSPNGFQESPPGVLSLRLSEPLVTKNGEITLKLGEGVDLDSSGKLISNTATKAAAPLSFSNNTISLNMDHPFYTKDGKLSLQVSPPLNILRTSILNTLALGFGSGLGLRGSALAVQLVSPLTFDTDGNIKLTLDRGLHVTTGDAIESNISWAKGLKFEDGAIATNIGNGLEFGSSSTETGVDDAYPIQVKLGSGLSFDSTGAIMAGNKEDDKLTLWTTPDPSPNCQILAENDAKLTLCLTKCGSQILATVSVLVVGSGNLNPITGTVSSAQVFLRFDANGVLLTEHSTLKKYWGYRQGDSIDGTPYTNAVGFMPNLKAYPKSQSSTTKNNIVGQVYMNGDVSKPMLLTITLNGTDDSNSTYSMSFSYTWTNGSYVGATFGANSYTFSYIAQEKKKKKKK

SEQ ID NO: 65 - protein, 441 aa, synthetic construct
  REGION 1..441: note = Fiber Polypeptide
MKRARPSEDTFNPVYPYDTETGPPTVPFLTPPFVSPNGFQESPPGVLSLRLSEPLVTKNGEITLKLGEGVDLDSSGKLISNTATKAAAPLSFSNNTISLNMDHPFYTKDGKLSLQVSPPLNILRTSILNTLALGFGSGLGLRGSALAVQLVSPLTFDTDGNIKLTLDRGLHVTTGDAIESNISWAKGLKFEDGAIATNIGNGLEFGSSSTETGVDDAYPIQVKLGSGLSFDSTGAIMAGNKEDDKLTLWTTPDPSPNCQILAENDAKLTLCLTKCGSQILATVSVLVVGSGNLNPITGTVSSAQVFLRFDANGVLLTEHSTLKKYWGYRQGDSIDGTPYTNAVGFMPNLKAYPKSQSSTTKNNIVGQVYMNGDVSKPMLLTITLNGTDDSGGSSGKKKKKKKASGGSSTYSMSFSYTWTNGSYVGATFGANSYTFSYIAQE

SEQ ID NO: 66 - protein, 27 aa, Mus musculus
PVTLTITLTARGEHKEEELIGAYYSMS

SEQ ID NO: 67 - protein, 27 aa, Mus musculus
PVTLTITLLRQTGAASAVWGGAYYSMS

SEQ ID NO: 68 - protein, 23 aa, Adenovirus type 5
EMQFFSTTEATAGNGDNLTPKVV

SEQ ID NO: 69 - protein, 26 aa, synthetic construct
  REGION 1..26: note = Artificial Sequence
EMQFFSGSTARGEHKEEELIGTPKVV

SEQ ID NO: 70 - protein, 27 aa, synthetic construct
  REGION 1..27: note = Artificial Sequence
EMQFFSGSMLRQTGAASAVWGGTPKVV

SEQ ID NO: 71 - protein, 407 aa, Adenovirus type 5
YNALAPKGAPNPCEWDEAATALEINLEEEDDDNEDEVDEQAEQQKTHVFSQAPYSGINITKEGIQIGVEGQTPKYADKTFQPEPQIGESQWYETEINHAAGRVLKKTTPMKPCYGSYAKPTNENGGQGILVKQQNGKLESQVEMQFFSTTEATAGNGDNLTPKVVLYSEDVDIETPDTHISYMPTIKEGNSRELMGQQSMPNRPNYIAFRDNFIGLMYYNSTGNMGVLAGQASQLNAVVDLQDRNTELSYQLLLDSIGDRTRYFSMWNQAVDSYDPDVRIIENHGTEDELPNYCFPLGGVINTETLTKVKPKTGQENGWEKDATEFSDKNEIRVGNNFAMEINLNANLWRNFLYSNIALYLPDKLKYSPSNVKISDNPNTYDYMNKRVVAPGLVDCYINLGARWSLD

SEQ ID NO: 72 - protein, 418 aa, Adenovirus type 6
YNALAPKGAPNSCEWEQNETAQVDAQELDEEENEANEAQAREQEQAKKTHVYAQAPLSGIKITKEGLQIGTADATVAGAGKEIFADKTFQPEPQVGESQWNEADATAAGGRVLKKTTPMKPCYGSYARPTNSNGGQGVMVEQNGKLESQVEMQFFSTSTNATNEVNNIQPTVVLYSEDVNMETPDTHLSYKPKMGDKNAKVMLGQQAMPNRPNYIAFRDNFIGLMYYNSTGNMGVLAGQASQLNAVVDLQDRNTELSYQLLLDSIGDRTRYFSMWNQAVDSYDPDVRIIENHGTEDELPNYCFPLGGIGITDTFQAVKTTAANGDQGNTTWQKDSTFAERNEIGVGNNFAMEINLNANLWRNFLYSNIALYLPDKLKYNPTNVEISDNPNTYDYMNKRVVAPGLVDCYINLGARWSLE

SEQ ID NO: 73 - protein, 414 aa, Adenovirus type 57
YNALAPKGAPNSCEWDEDDTQVQVAAEDDQDDDEEEEQLPQQRNGKKTHVYAQAPFAGEAINKNGLQIGTNGAATEGNKEIYADKTYQPEPQIGESQWNEAESSVAGGRVLKKTTPMKPCYGSYARPTNSNGGQGVMVEQNGKLESQVEMQFFSTSVNAMNEANAIQPKLVLYSEDVNMETPDTHLSYKPGKSDDNSKAMLGQQSMPNRPNYIAFRDNFIGLMYYNSTGNMGVLAGQASQLNAVVDLQDRNTELSYQLLLDSIGDRTRYFSMWNQAVDSYDPDVRIIENHGTEDELPNYCFPLGGIGVTDTYQAIKATNGNGGATTWAQDNTFAERNEIGVGNNFAMEINLNANLWRNFLYSNIALYLPDKLKYNPTNVEISDNPNTYDYMNKRVVAPGLVDCYINLGARWSLD

SEQ ID NO: 74 - protein, 348 aa, Adenovirus type 1
YNALAPKGAPNSCEWEQEEPTQEMAEELEDEEEAEEEEAEEEAEAPQADQKVKKTHVYAQAPLAGEKITANGLQIVSDTQTEGNPVFADPTYQPEPQVGESQWNEAEATASGGRVLKKTTPMKPCYGSYARPTNKNGGQGILVANNQGALESKVEMQFFAPSGTAMNERNAVQPSIVLYSEDVNMETPDTHISYKPSKTDENSKAMLGQQAMPNRPNYIAFRDNFIGLMYYNSTGNMGVLAGQASQLNAVVDLQDRNTELSYQLLLDSIGDRTRYFSMWNQAVDSYDPDVRIIENHGTEDELPNYCFPLGGIGVTDTYQGIKSNGNGNPQNWTKNDDFAARNEIGVGN

SEQ ID NO: 75 - protein, 352 aa, Adenovirus type 2
YNALAPKGAPNSCEWEQTEDSGRAVAEDEEEEDEDEEEEEEEQNARDQATKKTHVYAQAPLSGETITKSGLQIGSDNAETQAKPVYADPSYQPEPQIGESQWNEADANAAGGRVLKKTTPMKPCYGSYARPTNPFGGQSVLVPDEKGVPLPKVDLQFFSNTTSLNDRQGNATKPKVVLYSEDVNMETPDTHLSYKPGKGDENSKAMLGQQSMPNRPNYIAFRDNFIGLMYYNSTGNMGVLAGQASQLNAVVDLQDRNTELSYQLLLDSIGDRTRYFSMWNQAVDSYDPDVRIIENHGTEDELPNYCFPLGGIGVTDTYQAIKANGNGSGDNGDTTWTKDETFATRNEIGVGN

SEQ ID NO: 76 - protein, 336 aa, Adenovirus type 5
YNALAPKGAPNPCEWDEAATALEINLEEEDDDNEDEVDEQAEQQKTHVFSQAPYSGINITKEGIQIGVEGQTPKYADKTFQPEPQIGESQWYETEINHAAGRVLKKTTPMKPCYGSYAKPTNENGGQGILVKQQNGKLESQVEMQFFSTTEATAGNGDNLTPKVVLYSEDVDIETPDTHISYMPTIKEGNSRELMGQQSMPNRPNYIAFRDNFIGLMYYNSTGNMGVLAGQASQLNAVVDLQDRNTELSYQLLLDSIGDRTRYFSMWNQAVDSYDPDVRIIENHGTEDELPNYCFPLGGVINTETLTKVKPKTGQENGWEKDATEFSDKNEIRVGN

SEQ ID NO: 77 - protein, 347 aa, Adenovirus type 6
YNALAPKGAPNSCEWEQNETAQVDAQELDEEENEANEAQAREQEQAKKTHVYAQAPLSGIKITKEGLQIGTADATVAGAGKEIFADKTFQPEPQVGESQWNEADATAAGGRVLKKTTPMKPCYGSYARPTNSNGGQGVMVEQNGKLESQVEMQFFSTSTNATNEVNNIQPTVVLYSEDVNMETPDTHLSYKPKMGDKNAKVMLGQQAMPNRPNYIAFRDNFIGLMYYNSTGNMGVLAGQASQLNAVVDLQDRNTELSYQLLLDSIGDRTRYFSMWNQAVDSYDPDVRIIENHGTEDELPNYCFPLGGIGITDTFQAVKTTAANGDQGNTTWQKDSTFAERNEIGVGN

SEQ ID NO: 78 - protein, 343 aa, Adenovirus type 57
YNALAPKGAPNSCEWDEDDTQVQVAAEDDQDDDEEEEQLPQQRNGKKTHVYAQAPFAGEAINKNGLQIGTNGAATEGNKEIYADKTYQPEPQIGESQWNEAESSVAGGRVLKKTTPMKPCYGSYARPTNSNGGQGVMVEQNGKLESQVEMQFFSTSVNAMNEANAIQPKLVLYSEDVNMETPDTHLSYKPGKSDDNSKAMLGQQSMPNRPNYIAFRDNFIGLMYYNSTGNMGVLAGQASQLNAVVDLQDRNTELSYQLLLDSIGDRTRYFSMWNQAVDSYDPDVRIIENHGTEDELPNYCFPLGGIGVTDTYQAIKATNGNGGATTWAQDNTFAERNEIGVGN